European Patent Specification EP 3 479 844 B1, published November 22, 2023. Title: COVALENT DIABODIES AND USES THEREOF. Applicant: MacroGenics, Inc. The sequence listing filed with the application follows.

SEQUENCE LISTING (104 sequences)

SEQ ID NO: 1 - protein, 13 aa, Homo sapiens
  human IgG1 hinge
EPKSCDKTHTCPP

SEQ ID NO: 2 - protein, 10 aa, Homo sapiens
  human IgG2 hinge
ERKCCVECPP

SEQ ID NO: 3 - protein, 60 aa, Homo sapiens
  human IgG3 hinge
ELKTPLGDTTHTCPRCPEPKSCDTPPPCPRCPEPKSCDTPPPCPRCPEPKSCDTPPPCPR

SEQ ID NO: 4 - protein, 10 aa, Homo sapiens
  human IgG4 hinge
ESKYGPPCPS

SEQ ID NO: 5 - protein, 217 aa, Homo sapiens
  human IgG1 Fc domain
APELLGGPSVFLFPPKPKDTLMISRTPEVTCVVVDVSHEDPEVKFNWYVDGVEVHNAKTKPREEQYNSTYRVVSVLTVLHQDWLNGKEYKCKVSNKALPAPIEKTISKAKGQPREPQVYTLPPSRDELTKNQVSLTCLVKGFYPSDIAVEWESNGQPENNYKTTPPVLDSDGSFFLYSKLTVDKSRWQQGNVFSCSVMHEALHNHYTQKSLSLSPGK

SEQ ID NO: 6 - protein, 216 aa, Homo sapiens
  human IgG2 Fc domain
APPVAGPSVFLFPPKPKDTLMISRTPEVTCVVVDVSHEDPEVQFNWYVDGVEVHNAKTKPREEQFNSTFRVVSVLTVVHQDWLNGKEYKCKVSNKGLPAPIEKTISKTKGQPREPQVYTLPPSREEMTKNQVSLTCLVKGFYPSDIAVEWESNGQPENNYKTTPPMLDSDGSFFLYSKLTVDKSRWQQGNVFSCSVMHEALHNHYTQKSLSLSPGK

SEQ ID NO: 7 - protein, 217 aa, Homo sapiens
  human IgG3 Fc domain
APELLGGPSVFLFPPKPKDTLMISRTPEVTCVVVDVSHEDPEVQFKWYVDGVQVHNAKTKPREQQFNSTFRVVSVLTVLHQNWLDGKEYKCKVSNKALPAPIEKTISKTKGQPREPQVYTLPPSREEMTKNQVSLTCLVKGFYPSDIAVEWESSGQPENNYNTTPPMLDSDGSFFLYSKLTVDKSRWQQGNIFSCSVMHEALHNRFTQKSLSLSPGK

SEQ ID NO: 8 - protein, 217 aa, Homo sapiens
  human IgG4 Fc domain
APEFLGGPSVFLFPPKPKDTLMISRTPEVTCVVVDVSQEDPEVQFNWYVDGVEVHNAKTKPREEQFNSTYRVVSVLTVLHQDWLNGKEYKCKVSNKGLPSSIEKTISKAKGQPREPQVYTLPPSQEEMTKNQVSLTCLVKGFYPSDIAVEWESNGQPENNYKTTPPVLDSDGSFFLYSRLTVDKSRWQEGNVFSCSVMHEALHNHYTQKSLSLSLGK

SEQ ID NO: 9 - protein, 237 aa, Artificial Sequence
  Diabody Construct 1
EIVLTQSPDFQSVTPKEKVTFTCRTSQSIGTNIHWYQQKPDQSPKLLIKEVSESISGVPSRFSGSGSGTDFTLTINSLEAEDAATYYCQQSNTWPFTFGGGTKVEIKGGGSGGGGQVTLRESGPALVKPTQTLTLTCTFSGFSLSTSGMGVGWIRQPPGKALEWLAHIWWDDDKRYNPALKSRLTISKDTSKNQVVLTMTNMDPVDTATYYCAQINPAWFAYWGQGTLVTVSSLGGC

SEQ ID NO: 10 - protein, 8 aa, Artificial Sequence
  linker
GGGSGGGG

SEQ ID NO: 11 - protein, 244 aa, Artificial Sequence
  Diabody Construct 2
DIVMTQSPDSLAVSLGERATINCKASQSVDFDGDSFMNWYQQKPGQPPKLLIYTTSNLESGVPDRFSGSGSGTDFTLTISSLQAEDVAVYYCQQSNEDPYTFGQGTKLEIKGGGSGGGGQVQLVQSGAEVKKPGASVKVSCKASGYTFTNYWIHWVRQAPGQGLEWIGVIDPSDTYPNYNKKFKGRVTMTVVVSTSTAYMELRSLRSDDTAVYYCARNGDSDYYSGMDYWGQGTTVTVSSLGGC

SEQ ID NO: 12 - protein, 240 aa, Artificial Sequence
  Diabody Construct 3
EIVLTQSPDFQSVTPKEKVTFTCRTSQSIGTNIHWYQQKPDQSPKLLIKEVSESISGVPSRFSGSGSGTDFTLTINSLEAEDAATYYCQQSNTWPFTFGGGTKVEIKGGGSGGGGQVQLVQSGAEVKKPGASVKVSCKASGYTFTNYWIHWVRQAPGQGLEWIGVIDPSDTYPNYNKKFKGRVTMTVVVSTSTAYMELRSLRSDDTAVYYCARNGDSDYYSGMDYWGQGTTVTVSSLGGC

SEQ ID NO: 13 - protein, 241 aa, Artificial Sequence
  Diabody Construct 4
DIVMTQSPDSLAVSLGERATINCKASQSVDFDGDSFMNWYQQKPGQPPKLLIYTTSNLESGVPDRFSGSGSGTDFTLTISSLQAEDVAVYYCQQSNEDPYTFGQGTKLEIKGGGSGGGGQVTLRESGPALVKPTQTLTLTCTFSGFSLSTSGMGVGWIRQPPGKALEWLAHIWWDDDKRYNPALKSRLTISKDTSKNQVVLTMTNMDPVDTATYYCAQINPAWFAYWGQGTLVTVSSLGGC

SEQ ID NO: 14 - protein, 470 aa, Artificial Sequence
  Diabody Construct 5
EIVLTQSPDFQSVTPKEKVTFTCRTSQSIGTNIHWYQQKPDQSPKLLIKEVSESISGVPSRFSGSGSGTDFTLTINSLEAEDAATYYCQQSNTWPFTFGGGTKVEIKGGGSGGGGQVTLRESGPALVKPTQTLTLTCTFSGFSLSTSGMGVGWIRQPPGKALEWLAHIWWDDDKRYNPALKSRLTISKDTSKNQVVLTMTNMDPVDTATYYCAQINPAWFAYWGQGTLVTVSSLGGCVEPKSCDKTHTCPPCPAPELLGGPSVFLFPPKPKDTLMISRTPEVTCVVVDVSHEDPEVKFNWYVDGVEVHNAKTKPREEQYNSTYRVVSVLTVLHQDWLNGKEYKCKVSNKALPAPIEKTISKAKGQPREPQVYTLPPSRDELTKNQVSLTCLVKGFYPSDIAVEWESNGQPENNYKTTPPVLDSDGSFFLYSKLTVDKSRWQQGNVFSCSVMHEALHNHYTQKSLSLSPGK

SEQ ID NO: 15 - protein, 477 aa, Artificial Sequence
  Diabody Construct 6
DIVMTQSPDSLAVSLGERATINCKASQSVDFDGDSFMNWYQQKPGQPPKLLIYTTSNLESGVPDRFSGSGSGTDFTLTISSLQAEDVAVYYCQQSNEDPYTFGQGTKLEIKGGGSGGGGQVQLVQSGAEVKKPGASVKVSCKASGYTFTNYWIHWVRQAPGQGLEWIGVIDPSDTYPNYNKKFKGRVTMTVVVSTSTAYMELRSLRSDDTAVYYCARNGDSDYYSGMDYWGQGTTVTVSSLGGCVEPKSCDKTHTCPPCPAPELLGGPSVFLFPPKPKDTLMISRTPEVTCVVVDVSHEDPEVKFNWYVDGVEVHNAKTKPREEQYNSTYRVVSVLTVLHQDWLNGKEYKCKVSNKALPAPIEKTISKAKGQPREPQVYTLPPSRDELTKNQVSLTCLVKGFYPSDIAVEWESNGQPENNYKTTPPVLDSDGSFFLYSKLTVDKSRWQQGNVFSCSVMHEALHNHYTQKSLSLSPGK

SEQ ID NO: 16 - protein, 243 aa, Artificial Sequence
  Diabody Construct 7
EIVLTQSPDFQSVTPKEKVTFTCRTSQSIGTNIHWYQQKPDQSPKLLIKEVSESISGVPSRFSGSGSGTDFTLTINSLEAEDAATYYCQQSNTWPFTFGGGTKVEIKGGGSGGGGQVTLRESGPALVKPTQTLTLTCTFSGFSLSTSGMGVGWIRQPPGKALEWLAHIWWDDDKRYNPALKSRLTISKDTSKNQVVLTMTNMDPVDTATYYCAQINPAWFAYWGQGTLVTVSSLGGCFNRGEC

SEQ ID NO: 17 - protein, 10 aa, Artificial Sequence
  Linker plus C-terminus of human IgG-kappa chain
LGGCFNRGEC

SEQ ID NO: 18 - protein, 477 aa, Artificial Sequence
  Diabody Construct 8
DIVMTQSPDSLAVSLGERATINCKASQSVDFDGDSFMNWYQQKPGQPPKLLIYTTSNLESGVPDRFSGSGSGTDFTLTISSLQAEDVAVYYCQQSNEDPYTFGQGTKLEIKGGGSGGGGQVQLVQSGAEVKKPGASVKVSCKASGYTFTNYWIHWVRQAPGQGLEWIGVIDPSDTYPNYNKKFKGRVTMTVVVSTSTAYMELRSLRSDDTAVYYCARNGDSDYYSGMDYWGQGTTVTVSSLGGCAEPKSCDKTHTCPPCPAPELLGGPSVFLFPPKPKDTLMISRTPEVTCVVVDVSHEDPEVKFNWYVDGVEVHNAKTKPREEQYNSTYRVVSVLTVLHQDWLNGKEYKCKVSNKALPAPIEKTISKAKGQPREPQVYTLPPSRDELTKNQVSLTCLVKGFYPSDIAVEWESNGQPENNYKTTPPVLDSDGSFFLYSKLTVDKSRWQQGNVFSCSVMHEALHNHYTQKSLSLSPGK

SEQ ID NO: 19 - protein, 485 aa, Artificial Sequence
  Diabody Construct 9
VEPKSCDKTHTCPPCPAPELLGGPSVFLFPPKPKDTLMISRTPEVTCVVVDVSHEDPEVKFNWYVDGVEVHNAKTKPREEQYNSTYRVVSVLTVLHQDWLNGKEYKCKVSNKALPAPIEKTISKAKGQPREPQVYTLPPSRDELTKNQVSLTCLVKGFYPSDIAVEWESNGQPENNYKTTPPVLDSDGSFFLYSKLTVDKSRWQQGNVFSCSVMHEALHNHYTQKSLSLSPGKGGGSGGGGDIVMTQSPDSLAVSLGERATINCKASQSVDFDGDSFMNWYQQKPGQPPKLLIYTTSNLESGVPDRFSGSGSGTDFTLTISSLQAEDVAVYYCQQSNEDPYTFGQGTKLEIKGGGSGGGGQVQLVQSGAEVKKPGASVKVSCKASGYTFTNYWIHWVRQAPGQGLEWIGVIDPSDTYPNYNKKFKGRVTMTVVVSTSTAYMELRSLRSDDTAVYYCARNGDSDYYSGMDYWGQGTTVTVSSLGGC

SEQ ID NO: 20 - protein, 469 aa, Artificial Sequence
  Diabody Construct 10
APELLGGPSVFLFPPKPKDTLMISRTPEVTCVVVDVSHEDPEVKFNWYVDGVEVHNAKTKPREEQYNSTYRVVSVLTVLHQDWLNGKEYKCKVSNKALPAPIEKTISKAKGQPREPQVYTLPPSRDELTKNQVSLTCLVKGFYPSDIAVEWESNGQPENNYKTTPPVLDSDGSFFLYSKLTVDKSRWQQGNVFSCSVMHEALHNHYTQKSLSLSPGKGGGSGGGGDIVMTQSPDSLAVSLGERATINCKASQSVDFDGDSFMNWYQQKPGQPPKLLIYTTSNLESGVPDRFSGSGSGTDFTLTISSLQAEDVAVYYCQQSNEDPYTFGQGTKLEIKGGGSGGGGQVQLVQSGAEVKKPGASVKVSCKASGYTFTNYWIHWVRQAPGQGLEWIGVIDPSDTYPNYNKKFKGRVTMTVVVSTSTAYMELRSLRSDDTAVYYCARNGDSDYYSGMDYWGQGTTVTVSSLGGC

SEQ ID NO: 21 - protein, 466 aa, Artificial Sequence
  Diabody Construct 11
EIVLTQSPDFQSVTPKEKVTFTCRTSQSIGTNIHWYQQKPDQSPKLLIKEVSESISGVPSRFSGSGSGTDFTLTINSLEAEDAATYYCQQSNTWPFTFGCGTKVEIKGGGSGGGGQVTLRESGPALVKPTQTLTLTCTFSGFSLSTSGMGVGWIRQPPGKALEWLAHIWWDDDKRYNPALKSRLTISKDTSKNQVVLTMTNMDPVDTATYYCAQINPAWFAYWGQGTLVTVSSVEPKSCDKTHTCPPCPAPELLGGPSVFLFPPKPKDTLMISRTPEVTCVVVDVSHEDPEVKFNWYVDGVEVHNAKTKPREEQYNSTYRVVSVLTVLHQDWLNGKEYKCKVSNKALPAPIEKTISKAKGQPREPQVYTLPPSRDELTKNQVSLTCLVKGFYPSDIAVEWESNGQPENNYKTTPPVLDSDGSFFLYSKLTVDKSRWQQGNVFSCSVMHEALHNHYTQKSLSLSPGK

SEQ ID NO: 22 - protein, 246 aa, Artificial Sequence
  Diabody Construct 12
DIVMTQSPDSLAVSLGERATINCKASQSVDFDGDSFMNWYQQKPGQPPKLLIYTTSNLESGVPDRFSGSGSGTDFTLTISSLQAEDVAVYYCQQSNEDPYTFGQGTKLEIKGGGSGGGGQVQLVQSGAEVKKPGASVKVSCKASGYTFTNYWIHWVRQAPGQCLEWIGVIDPSDTYPNYNKKFKGRVTMTVVVSTSTAYMELRSLRSDDTAVYYCARNGDSDYYSGMDYWGQGTTVTVSSFNRGEC

SEQ ID NO: 23 - protein, 6 aa, Homo sapiens
  C-terminus of human IgG Kappa chain
FNRGEC

SEQ ID NO: 24 - protein, 5 aa, Artificial Sequence
  2B6 Heavy chain variable region - CDR1
NYWIH

SEQ ID NO: 25 - protein, 5 aa, Artificial Sequence
  3H7 Heavy Chian Variable region - CDR1
DAWMD

SEQ ID NO: 26 - protein, 17 aa, Artificial Sequence
  2B6 Heavy chain variable region - CDR2
VIDPSDTYPNYNKKFKG

SEQ ID NO: 27 - protein, 19 aa, Artificial Sequence
  3H7 Heavy Chian Variable region - CDR2
EIRNKANNLATYYAESVKG

SEQ ID NO: 28 - protein, 12 aa, Artificial Sequence
  2B6 Heavy chain variable region - CDR3
NGDSDYYSGMDY

SEQ ID NO: 29 - protein, 6 aa, Artificial Sequence
  3H7 Heavy Chian Variable region - CDR3
YSPFAY

SEQ ID NO: 30-31 - skipped (2 entries)

SEQ ID NO: 32 - protein, 11 aa, Artificial Sequence
  2B6 Light chain variable region - CDR1
RTSQSIGTNIH

SEQ ID NO: 33 - protein, 11 aa, Artificial Sequence
  3H7 Light Chian Variable region - CDR1
RASQEISGYLS

SEQ ID NO: 34 - protein, 7 aa, Artificial Sequence
  2B6 Light chain variable region - CDR2
NVSESIS

SEQ ID NO: 35 - protein, 7 aa, Artificial Sequence
  2B6 Light chain variable region - CDR2
YVSESIS

SEQ ID NO: 36 - protein, 7 aa, Artificial Sequence
  2B6 Light chain variable region - CDR2
YASESIS

SEQ ID NO: 37 - protein, 7 aa, Artificial Sequence
  3H7 Light Chian Variable region - CDR2
AASTLDS

SEQ ID NO: 38 - protein, 9 aa, Artificial Sequence
  2B6 Light chain variable region - CDR3
QQSNTWPFT

SEQ ID NO: 39 - protein, 9 aa, Artificial Sequence
  3H7 Light Chian Variable region - CDR3
LQYVSYPYT

SEQ ID NO: 40 - protein, 121 aa, Artificial Sequence
  2B6 heavy chain variable region
QVQLVQSGAEVKKPGASVKVSCKASGYTFTNYWIHWVRQAPGQGLEWMGVIDPSDTYPNYNKKFKGRVTMTTDTSTSTAYMELRSLRSDDTAVYYCARNGDSDYYSGMDYWGQGTTVTVSS

SEQ ID NO: 41 - protein, 107 aa, Artificial Sequence
  2B6 light chain variable region - Hu2B6VL-1
EIVLTQSPDFQSVTPKEKVTITCRTSQSIGTNIHWYQQKPDQSPKLLIKNVSESISGVPSRFSGSGSGTDFTLTINSLEAEDAATYYCQQSNTWPFTFGGGTKVEIK

SEQ ID NO: 42 - protein, 107 aa, Artificial Sequence
  Humanized 2B6 light chain variable region - Hu2B6VL-2
EIVLTQSPDFQSVTPKEKVTITCRTSQSIGTNIHWYQQKPDQSPKLLIKYVSESISGVPSRFSGSGSGTDFTLTINSLEAEDAATYYCQQSNTWPFTFGGGTKVEIK

SEQ ID NO: 43 - protein, 107 aa, Artificial Sequence
  Humanized 2B6 light chain variable region - Hu2B6VL-3
EIVLTQSPDFQSVTPKEKVTITCRTSQSIGTNIHWYQQKPDQSPKLLIKYASESISGVPSRFSGSGSGTDFTLTINSLEAEDAATYYCQQSNTWPFTFGGGTKVEIK

SEQ ID NO: 44 - protein, 107 aa, mus sp.
  mouse 3H7 Light Chain Variable Region
DIQMTQSPSSLSASLGERVSLTCRASQEISGYLSWLQQKPDGTIRRLIYAASTLDSGVPKRFSGSWSGSDYSLTISSLESEDFADYYCLQYVSYPYTFGGGTKLEIK

SEQ ID NO: 45 - protein, 9 aa, Artificial Sequence
  IgG binding site of the Fc-gamma-RIIB receptor
KKFSRSDPN

SEQ ID NO: 46 - protein, 9 aa, Artificial Sequence
  IgG binding site of the Fc-gamma-RIIB receptor
QKFSRLDPN

SEQ ID NO: 47 - protein, 9 aa, Artificial Sequence
  IgG binding site of the Fc-gamma-RIIB receptor
QKFSRLDPT

SEQ ID NO: 48 - protein, 9 aa, Artificial Sequence
  IgG binding site of the Fc-gamma-RIIB receptor
KKFSRLDPT

SEQ ID NO: 49 - protein, 9 aa, Artificial Sequence
  IgG binding site of the Fc-gamma-RIIB receptor
QKFSHLDPT

SEQ ID NO: 50 - protein, 9 aa, Artificial Sequence
  IgG binding site of the Fc-gamma-RIIB receptor
KKFSHLDPT

SEQ ID NO: 51 - protein, 9 aa, Artificial Sequence
  IgG binding site of the Fc-gamma-RIIB receptor
QKFSRLDPN

SEQ ID NO: 52 - protein, 9 aa, Artificial Sequence
  IgG binding site of the Fc-gamma-RIIB receptor
KKFSRSDPN

SEQ ID NO: 53 - protein, 9 aa, Artificial Sequence
  IgG binding site of the Fc-gamma-RIIB receptor
QKFSRLDPT

SEQ ID NO: 54 - protein, 9 aa, Artificial Sequence
  IgG binding site of the Fc-gamma-RIIB receptor
QKFSHLDPT

SEQ ID NO: 55 - protein, 9 aa, Artificial Sequence
  IgG binding site of the Fc-gamma-RIIB receptor
KKFSRLDPT

SEQ ID NO: 56 - protein, 9 aa, Artificial Sequence
  IgG binding site of the Fc-gamma-RIIB receptor
KKFSHLDPT

SEQ ID NO: 57 - DNA, 36 bp, Artificial Sequence
  Lgh321F primer
cgagctagctctagatgagatcacagttctctctac

SEQ ID NO: 58 - DNA, 47 bp, Artificial Sequence
  Lgh318R primer
gcctccgcctccggatccgcctcctttgatctccaccttggtccctc

SEQ ID NO: 59 - DNA, 47 bp, Artificial Sequence
  Lgh319F primer
ggaggcggatccggaggcggaggccaggttcagctggtgcagtctgg

SEQ ID NO: 60 - DNA, 43 bp, Artificial Sequence
  Lgh320R primer
tttgaattctagcagcctcccagtgaggagacggtgaccgtgg

SEQ ID NO: 61 - DNA, 46 bp, Artificial Sequence
  Lgh315R primer
gcctccgcctccggatccgcctcctttgatctcaagcttggtcccc

SEQ ID NO: 62 - DNA, 48 bp, Artificial Sequence
  Lgh316F primer
ggaggcggatccggaggcggaggccaggttaccctgagagagtctggc

SEQ ID NO: 63 - DNA, 47 bp, Artificial Sequence
  Lgh317R primer
tttgaattcctagcagcctcccagtgagctcacagtgaccagagtcc

SEQ ID NO: 64 - DNA, 27 bp, Artificial Sequence
  Lgh339R primer
ctcaacgcagcctcccagtgagctcac

SEQ ID NO: 65 - DNA, 31 bp, Artificial Sequence
  Lgh340R primer
aacgcagcctcccagtgaggagacggtgacc

SEQ ID NO: 66 - DNA, 27 bp, Artificial Sequence
  Lgh366R primer
tttgaattctatttacccggagacagg

SEQ ID NO: 67 - DNA, 33 bp, Artificial Sequence
  Lgh367F primer
ctgggaggctgcgcagagcccaaatcttgtgac

SEQ ID NO: 68 - DNA, 33 bp, Artificial Sequence
  Lgh368R primer
gtcacaagatttgggctctgcgcagcctcccag

SEQ ID NO: 69 - DNA, 50 bp, Artificial Sequence
  Lgh369R primer
tttgaattctaacactctcccctgttgaagcagcctcccagtgaggagac

SEQ ID NO: 70 - protein, 118 aa, Artificial Sequence
  humanized anti-CD16A heavy chain variable region(Hu3G8VH-1)
QVTLRESGPALVKPTQTLTLTCTFSGFSLSTSGMGVGWIRQPPGKALEWLAHIWWDDDKRYNPALKSRLTISKDTSKNQVVLTMTNMDPVDTATYYCARINPAWFAYWGQGTLVTVSS

SEQ ID NO: 71 - protein, 118 aa, Artificial Sequence
  humanized anti-CD16A heavy chain variable region(Hu3G8VH-5)
QVTLRESGPALVKPTQTLTLTCTFSGFSLSTSGMGVGWIRQPPGKALEWLAHIWWDDDKRYNPALKSRLTISKDTSKNQVVLTMTNMDPVDTATYYCAQINPAWFAYWGQGTLVTVSS

SEQ ID NO: 72 - protein, 117 aa, Artificial Sequence
  humanized anti-CD16A heavy chain variable region(Hu3G8VH-22)
QVTLRESGPALVKPTQTLTLTCTFSGFSLSTSGVGVGWIRQPPGKALEWLAHIWWDDDKRYSPSLKSRLTISKDTSKNQVVLTMTNMDPVDTATYYCARINPAYFAYWGQGTLVTVS

SEQ ID NO: 73 - protein, 111 aa, Artificial Sequence
  humanized anti-CD16A light chain variable region(Hu3G8VL-1)
DIVMTQSPDSLAVSLGERATINCKASQSVDFDGDSFMNWYQQKPGQPPKLLIYTTSNLESGVPDRFSGSGSGTDFTLTISSLQAEDVAVYYCQQSNEDPYTFGQGTKLEIK

SEQ ID NO: 74 - protein, 111 aa, Artificial Sequence
  humanized anti-CD16A light chain variable region(Hu3G8VL-43)
DIVMTQSPDSLAVSLGERATINCKSSQSVDFDGDSFMNWYQQKPGQPPKLLIYTTSSLESGVPDRFSGSGSGTDFTLTISSLQAEDVAVYYCQQSNSDPYTFGQGTKLEIK

SEQ ID NO: 75 - protein, 111 aa, Artificial Sequence
  humanized anti-CD16A light chain variable region(Hu3G8VL-22)
DIVMTQSPDSLAVSLGERATINCKSSQSVDFDGDSFMNWYQQKPGQPPKLLIYTTSNLETGVPDRFSGSGSGTDFTLTISSLQAEDVAVYYCQQSNSDPYTFGQGTKLEIK

SEQ ID NO: 76 - DNA, 24 bp, Artificial Sequence
  DNA sequence of linker (SEQ ID NO. 10)
ggaggcggatccggaggcggaggc

SEQ ID NO: 77 - DNA, 18 bp, Homo sapiens
  DNA sequence of C-terminus of human IgG Kappa chain
ttcaacaggggagagtgt

SEQ ID NO: 78 - DNA, 30 bp, Artificial Sequence
  Linker plus C-terminus of human IgG Kappa chain
ctgggaggctgcttcaacaggggagagtgt

SEQ ID NO: 79 - protein, 6 aa, Homo sapiens
  Human IgG hinge domain
VEPKSC

SEQ ID NO: 80 - DNA, 18 bp, Homo sapiens
  Human IgG hinge domain
gttgagcccaaatcttgt

SEQ ID NO: 81 - protein, 118 aa, Homo sapiens
  VH domain of 3G8 antibody
QVTLKESGPGILQPSQTLSLTCSFSGFSLRTSGMGVGWIRQPSGKGLEWLAHIWWDDDKRYNPALKSRLTISKDTSSNQVFLKIASVDTADTATYYCAQINPAWFAYWGQGTLVTVSS

SEQ ID NO: 82 - DNA, 354 bp, Homo sapiens
  VH domain of 3G8 antibody
caggttaccctgaaagagtctggccctgggatattgcagccctcccagaccctcagtctgacttgttctttctctgggttttcactgaggacttctggtatgggtgtaggctggattcgtcagccttcagggaagggtctagagtggctggcacacatttggtgggatgatgacaagcgctataatccagccctgaagagccgactgacaatctccaaggatacctccagcaaccaggtattcctcaaaatcgccagtgtggacactgcagatactgccacatactactgtgctcaaataaaccccgcctggtttgcttactggggccaagggactctggtcactgtgagctca

SEQ ID NO: 83 - DNA, 354 bp, Artificial Sequence
  humanized anti-CD16A heavy chain variable region(Hu3G8VH-5)
caggttaccctgagagagtctggccctgcgctggtgaagcccacacagaccctcacactgacttgtaccttctctgggttttcactgagcacttctggtatgggtgtaggctggattcgtcagcctcccgggaaggctctagagtggctggcacacatttggtgggatgatgacaagcgctataatccagccctgaagagccgactgacaatctccaaggatacctccaaaaaccaggtagtcctcacaatgaccaacatggaccctgtggatactgccacatactactgtgctcaaataaaccccgcctggtttgcttactggggccaagggactctggtcactgtgagctca

SEQ ID NO: 84 - protein, 111 aa, Homo sapiens
  VL domain of 3G8 antibody
DTVLTQSPASLAVSLGQRATISCKASQSVDFDGDSFMNWYQQKPGQPPKLLIYTTSNLESGIPARFSASGSGTDFTLNIHPVEEEDTATYYCQQSNEDPYTFGGGTKLEIK

SEQ ID NO: 85 - DNA, 333 bp, Homo sapiens
  VL domain of 3G8 antibody
gacactgtgctgacccaatctccagcttctttggctgtgtctctagggcagagggccaccatctcctgcaaggccagccaaagtgttgattttgatggtgatagttttatgaactggtaccaacagaaaccaggacagccacccaaactcctcatctatactacatccaatctagaatctgggatcccagccaggtttagtgccagtgggtctgggacagacttcaccctcaacatccatcctgtggaggaggaggatactgcaacctattactgtcagcaaagtaatgaggatccgtacacgttcggaggggggaccaagctggaaataaaa

SEQ ID NO: 86 - DNA, 333 bp, Artificial Sequence
  humanized anti-CD16A light chain variable region(Hu3G8VL-1)
gacatcgtgatgacccaatctccagactctttggctgtgtctctaggggagagggccaccatcaactgcaaggccagccaaagtgttgattttgatggtgatagttttatgaactggtaccaacagaaaccaggacagccacccaaactcctcatctatactacatccaatctagaatctggggtcccagacaggtttagtggcagtgggtctgggacagacttcaccctcaccatcagcagcctgcaggctgaggatgtggcagtttattactgtcagcaaagtaatgaggatccgtacacgttcggacaggggaccaagcttgagatcaaa

SEQ ID NO: 87 - protein, 121 aa, Artificial Sequence
  humanized 2B6 heavy chain variable region
QVQLVQSGAEVKKPGASVKVSCKASGYTFTNYWIHWVRQAPGQGLEWIGVIDPSDTYPNYNKKFKGRVTMTVVVSTSTAYMELRSLRSDDTAVYYCARNGDSDYYSGMDYWGQGTTVTVSS

SEQ ID NO: 88 - DNA, 363 bp, Artificial Sequence
  humanized 2B6 heavy chain variable region
caggttcagctggtgcagtctggagctgaggtgaagaagcctggggcctcagtgaaggtctcctgcaaggcttctggttacacctttaccaactactggatacactgggtgcgacaggcccctggacaagggcttgagtggattggagtgattgatccttctgatacttatccaaattacaataaaaagttcaagggcagagtcaccatgaccgtagtcgtatccacgagcacagcctacatggagctgaggagcctgagatctgacgacacggccgtgtattactgtgcgagaaacggtgattccgattattactctggtatggactactgggggcaagggaccacggtcaccgtctcctca

SEQ ID NO: 89 - protein, 111 aa, Artificial Sequence; identical to SEQ ID NO: 73
  humanized 2B6 light chain variable region

SEQ ID NO: 90 - DNA, 321 bp, Artificial Sequence
  humanized 2B6 light chain variable region
gaaattgtgctgactcagtctccagactttcagtctgtgactccaaaggagaaagtcaccttcacctgcaggaccagtcagagcattggcacaaacatacactggtaccagcagaaaccagatcagtctccaaagctcctcatcaaggaggtttctgagtctatctctggagtcccatcgaggttcagtggcagtggatctgggacagatttcaccctcaccatcaatagcctggaagctgaagatgctgcaacgtattactgtcaacaaagtaatacctggccgttcacgttcggcggagggaccaaggtggagatcaaa

SEQ ID NO: 91 - protein, 6 aa, Artificial Sequence
  thrombin cleavage recognition site
LVPRGS

SEQ ID NO: 92 - protein, 4 aa, Artificial Sequence
  Factor Xa cleavage recognition site
  VARIANT 2: Xaa = Glu or Asp
IXGR

SEQ ID NO: 93 - protein, 5 aa, Artificial Sequence
  enterokinase cleavage recognition site
DDDDK

SEQ ID NO: 94 - protein, 4 aa, Artificial Sequence
  furin cleavage recognition site
  VARIANT 2, 3: Xaa = Any Amino Acid
RXXR

SEQ ID NO: 95 - protein, 4 aa, Artificial Sequence
  preferred furin cleavage recognition site
  VARIANT 2: Xaa = Any Amino Acid
  VARIANT 3: Xaa = Lys or Arg
RXXR

SEQ ID NO: 96 - protein, 7 aa, Artificial Sequence
  AcTEV cleavage recognition site
ENLYFQG

SEQ ID NO: 97 - protein, 487 aa, Artificial Sequence
  covalent diabody polyprotein precursor (Construct 13)
DTVLTQSPASLAVSLGQRATISCKASQSVDFDGDSFMNWYQQKPGQPPKLLIYTTSNLESGIPARFSASGSGTDFTLNIHPVEEEDTATYYCQQSNEDPYTFGGGTKLEIKGGGSGGGGEVELVESGGGLVQPGRSLKLSCAASGFTFSDYYMAWVRQAPTTGLEWVASISYDGGDTHYRDSVKGRFTISRDNAKSSLYLQMDSLRSEDTATYYCATETTGIPTGVMDAWGQGVSVTVSSLGGCGGRAKRDVQMTQSPSNLAASPGESVSINCKASESISKYLAWYLQKPGKANKLLMYDGSTLQSGIPSRFSGSGSGTDFTLTIRSLEPEDFGLYYCQQHYEYPATFGSGTKLEIKGGGSGGGGQVTLKESGPGILQPSQTLSLTCSFSGFSLRTSGMGVGWIRQPSGKGLEWLAHIWWDDDKRYNPALKSRLTISKDTSSNQVFLKIASVDTADTATYYCAQINPAWFAYWGQGTLVTVSSLGGC

SEQ ID NO: 98 - DNA, 1464 bp, Artificial Sequence
  covalent diabody polyprotein precursor (DNA sequence of SEQ ID NO. 97)
gacactgtgctgacccaatctccagcttctttggctgtgtctctagggcagagggccaccatctcctgcaaggccagccaaagtgttgattttgatggtgatagttttatgaactggtaccaacagaaaccaggacagccacccaaactcctcatctatactacatccaatctagaatctgggatcccagccaggtttagtgccagtgggtctgggacagacttcaccctcaacatccatcctgtggaggaggaggatactgcaacctattactgtcagcaaagtaatgaggatccgtacacgttcggaggggggaccaagctggaaataaaaggaggcggatccggaggcggaggcgaggtggagctagtggagtctgggggaggcttagtgcagcctggaaggtccctgaaactctcgtgtgcagcctcaggattcactttcagtgactattacatggcctgggtccggcaggctccaacgacgggtctggagtgggtcgcatccattagttatgatggtggtgacactcactatcgagactccgtgaagggccgatttactatttccagagataatgcaaaaagcagcctatacctgcaaatggacagtctgaggtctgaggacacggccacttattactgtgcaacagagactacgggaatacctacaggtgttatggatgcctggggtcaaggagtttcagtcactgtctcctcactgggaggctgcggcgggagagctaagagggatgtccagatgacccagtctccatctaatcttgctgcctctcctggagaaagtgtttccatcaattgcaaggcaagtgagagcattagcaagtatttagcctggtatctacagaaacctgggaaagcaaataagcttcttatgtacgatgggtcaactttgcaatctggaattccatcgaggttcagtggcagtggatctggtacagatttcactctcaccatcagaagcctggagcctgaagattttggactctattactgtcaacagcattatgaatatccagccacgttcggttctgggaccaagctggagatcaaaggaggcggatccggaggcggaggccaggttaccctgaaagagtctggccctgggatattgcagccctcccagaccctcagtctgacttgttctttctctgggttttcactgaggacttctggtatgggtgtaggctggattcgtcagccttcagggaagggtctagagtggctggcacacatttggtgggatgatgacaagcgctataatccagccctgaagagccgactgacaatctccaaggatacctccagcaaccaggtattcctcaaaatcgccagtgtggacactgcagatactgccacatactactgtgctcaaataaaccccgcctggtttgcttactggggccaagggactctggtcactgtgagctcactgggaggctgctag

SEQ ID NO: 99 - protein, 511 aa, Artificial Sequence
  covalent diabody polyprotein precursor (Construct 14)
DTVLTQSPASLAVSLGQRATISCKASQSVDFDGDSFMNWYQQKPGQPPKLLIYTTSNLESGIPARFSASGSGTDFTLNIHPVEEEDTATYYCQQSNEDPYTFGGGTKLEIKGGGSGGGGEVELVESGGGLVQPGRSLKLSCAASGFTFSDYYMAWVRQAPTTGLEWVASISYDGGDTHYRDSVKGRFTISRDNAKSSLYLQMDSLRSEDTATYYCATETTGIPTGVMDAWGQGVSVTVSSLGGCGGRAKRAPVKQTLNFDLLKLAGDVESNPGPDVQMTQSPSNLAASPGESVSINCKASESISKYLAWYLQKPGKANKLLMYDGSTLQSGIPSRFSGSGSGTDFTLTIRSLEPEDFGLYYCQQHYEYPATFGSGTKLEIKGGGSGGGGQVTLKESGPGILQPSQTLSLTCSFSGFSLRTSGMGVGWIRQPSGKGLEWLAHIWWDDDKRYNPALKSRLTISKDTSSNQVFLKIASVDTADTATYYCAQINPAWFAYWGQGTLVTVSSLGGC

SEQ ID NO: 100 - DNA, 1536 bp, Artificial Sequence
  covalent diabody polyprotein precursor (DNA sequence of SEQ ID NO. 99)
gacactgtgctgacccaatctccagcttctttggctgtgtctctagggcagagggccaccatctcctgcaaggccagccaaagtgttgattttgatggtgatagttttatgaactggtaccaacagaaaccaggacagccacccaaactcctcatctatactacatccaatctagaatctgggatcccagccaggtttagtgccagtgggtctgggacagacttcaccctcaacatccatcctgtggaggaggaggatactgcaacctattactgtcagcaaagtaatgaggatccgtacacgttcggaggggggaccaagctggaaataaaaggaggcggatccggaggcggaggcgaggtggagctagtggagtctgggggaggcttagtgcagcctggaaggtccctgaaactctcgtgtgcagcctcaggattcactttcagtgactattacatggcctgggtccggcaggctccaacgacgggtctggagtgggtcgcatccattagttatgatggtggtgacactcactatcgagactccgtgaagggccgatttactatttccagagataatgcaaaaagcagcctatacctgcaaatggacagtctgaggtctgaggacacggccacttattactgtgcaacagagactacgggaatacctacaggtgttatggatgcctggggtcaaggagtttcagtcactgtctcctcactgggaggctgcggcgggagagctaagagggcccctgtgaagcagaccctgaacttcgacctgctgaagctggccggagacgtggagagcaaccccggccccgatgtccagatgacccagtctccatctaatcttgctgcctctcctggagaaagtgtttccatcaattgcaaggcaagtgagagcattagcaagtatttagcctggtatctacagaaacctgggaaagcaaataagcttcttatgtacgatgggtcaactttgcaatctggaattccatcgaggttcagtggcagtggatctggtacagatttcactctcaccatcagaagcctggagcctgaagattttggactctattactgtcaacagcattatgaatatccagccacgttcggttctgggaccaagctggagatcaaaggaggcggatccggaggcggaggccaggttaccctgaaagagtctggccctgggatattgcagccctcccagaccctcagtctgacttgttctttctctgggttttcactgaggacttctggtatgggtgtaggctggattcgtcagccttcagggaagggtctagagtggctggcacacatttggtgggatgatgacaagcgctataatccagccctgaagagccgactgacaatctccaaggatacctccagcaaccaggtattcctcaaaatcgccagtgtggacactgcagatactgccacatactactgtgctcaaataaaccccgcctggtttgcttactggggccaagggactctggtcactgtgagctcactgggaggctgctag

SEQ ID NO: 101 - protein, 239 aa, Artificial Sequence
  Diabody construct (Construct 15)
EIVLTQSPDFQSVTPKEKVTFTCRTSQSIGTNIHWYQQKPDQSPKLLIKEVSESISGVPSRFSGSGSGTDFTLTINSLEAEDAATYYCQQSNTWPFTFGGGTKVEIKGGGSGGGGQVTLRESGPALVKPTQTLTLTCTFSGFSLSTSGMGVGWIRQPPGKALEWLAHIWWDDDKRYNPALKSRLTISKDTSKNQVVLTMTNMDPVDTATYYCAQINPAWFAYWGQGTLVTVSSFNRGEC

SEQ ID NO: 102 - DNA, 720 bp, Artificial Sequence
  Diabody construct (DNA sequence of SEQ ID NO. 101)
gaaattgtgctgactcagtctccagactttcagtctgtgactccaaaggagaaagtcaccttcacctgcaggaccagtcagagcattggcacaaacatacactggtaccagcagaaaccagatcagtctccaaagctcctcatcaaggaggtttctgagtctatctctggagtcccatcgaggttcagtggcagtggatctgggacagatttcaccctcaccatcaatagcctggaagctgaagatgctgcaacgtattactgtcaacaaagtaatacctggccgttcacgttcggcggagggaccaaggtggagatcaaaggaggcggatccggaggcggaggccaggttaccctgagagagtctggccctgcgctggtgaagcccacacagaccctcacactgacttgtaccttctctgggttttcactgagcacttctggtatgggtgtaggctggattcgtcagcctcccgggaaggctctagagtggctggcacacatttggtgggatgatgacaagcgctataatccagccctgaagagccgactgacaatctccaaggatacctccaaaaaccaggtagtcctcacaatgaccaacatggaccctgtggatactgccacatactactgtgctcaaataaaccccgcctggtttgcttactggggccaagggactctggtcactgtgagctcattcaacaggggagagtgttag

SEQ ID NO: 103 - protein, 246 aa, Artificial Sequence
  Diabody construct (Construct 16)
DIVMTQSPDSLAVSLGERATINCKASQSVDFDGDSFMNWYQQKPGQPPKLLIYTTSNLESGVPDRFSGSGSGTDFTLTISSLQAEDVAVYYCQQSNEDPYTFGQGTKLEIKGGGSGGGGQVQLVQSGAEVKKPGASVKVSCKASGYTFTNYWIHWVRQAPGQGLEWIGVIDPSDTYPNYNKKFKGRVTMTVVVSTSTAYMELRSLRSDDTAVYYCARNGDSDYYSGMDYWGQGTTVTVSSVEPKSC

SEQ ID NO: 104 - DNA, 741 bp, Artificial Sequence
  Diabody construct (DNA sequence of SEQ ID NO. 103)
gacatcgtgatgacccaatctccagactctttggctgtgtctctaggggagagggccaccatcaactgcaaggccagccaaagtgttgattttgatggtgatagttttatgaactggtaccaacagaaaccaggacagccacccaaactcctcatctatactacatccaatctagaatctggggtcccagacaggtttagtggcagtgggtctgggacagacttcaccctcaccatcagcagcctgcaggctgaggatgtggcagtttattactgtcagcaaagtaatgaggatccgtacacgttcggacaggggaccaagcttgagatcaaaggaggcggatccggaggcggaggccaggttcagctggtgcagtctggagctgaggtgaagaagcctggggcctcagtgaaggtctcctgcaaggcttctggttacacctttaccaactactggatacactgggtgcgacaggcccctggacaagggcttgagtggattggagtgattgatccttctgatacttatccaaattacaataaaaagttcaagggcagagtcaccatgaccgtagtcgtatccacgagcacagcctacatggagctgaggagcctgagatctgacgacacggccgtgtattactgtgcgagaaacggtgattccgattattactctggtatggactactgggggcaagggaccacggtcaccgtctcctcagttgagcccaaatcttgttag